European Patent Application EP 4 273 232 A2, published November 8, 2023. Title: B-cell cultivation method. Applicant: F. Hoffmann-La Roche AG. The sequence listing filed with the application follows.

SEQUENCE LISTING (45 sequences)

SEQ ID NO: 1 - DNA, 32 bp, synthetic construct
  misc_feature 1..32: note = rb-V-kappa-HindIIIs primer
  source 1..32: mol_type = other DNA
gattaagcttatggacaygagggcccccactc

SEQ ID NO: 2 - DNA, 35 bp, synthetic construct
  misc_feature 1..35: note = rb-C-kappa-NheIas primer
  source 1..35: mol_type = other DNA
gatcgctagccctggcaggcgtctcrctctaacag

SEQ ID NO: 3 - DNA, 23 bp, synthetic construct
  misc_feature 1..23: note = rb-CH1rev-1 primer
  source 1..23: mol_type = other DNA
gcagggggccagtgggaagactg

SEQ ID NO: 4 - DNA, 29 bp, synthetic construct
  misc_feature 1..29: note = rbVH3-23for3 primer
  source 1..29: mol_type = other DNA
caccatggagactgggctgcgctggcttc

SEQ ID NO: 5 - DNA, 20 bp, synthetic construct
  misc_feature 1..20: note = bcPCR-huCgamma-rev primer
  source 1..20: mol_type = other DNA
cccccagaggtgctcttgga

SEQ ID NO: 6 - DNA, 20 bp, synthetic construct
  misc_feature 1..20: note = bcPCR-FHLC-leader-fw primer
  source 1..20: mol_type = other DNA
atggacatgagggtccccgc

SEQ ID NO: 7 - DNA, 24 bp, synthetic construct
  misc_feature 1..24: note = bcPCR-huCkappa-rev primer
  source 1..24: mol_type = other DNA
gatttcaactgctcatcagatggc

SEQ ID NO: 8 - DNA, 45 bp, synthetic construct
  misc_feature 1..45: note = bcPCR-hu-HC-10600-SLIC-as primer
  source 1..45: mol_type = other DNA
cagcccagtctccatggtggcaagcttcctctgtgttcagtgctg

SEQ ID NO: 9 - DNA, 26 bp, synthetic construct
  misc_feature 1..26: note = bcPCR-hu-HC-10600-SLIC-s primer
  source 1..26: mol_type = other DNA
ctccaagagcacctctgggggcacag

SEQ ID NO: 10 - DNA, 24 bp, synthetic construct
  misc_feature 1..24: note = bcPCR-hu-LC-10603-SLIC-s primer
  source 1..24: mol_type = other DNA
gccatctgatgagcagttgaaatc

SEQ ID NO: 11 - DNA, 38 bp, synthetic construct
  misc_feature 1..38: note = bcPCR-hu-LC-10603-SLIC-as primer
  source 1..38: mol_type = other DNA
gcggggaccctcatgtccatggtggcaagcttcctctg

SEQ ID NO: 12 - DNA, 48 bp, synthetic construct
  misc_feature 1..48: note = SLIC-hu-VHuniversal-for primer
  source 1..48: mol_type = other DNA
agcaacagctacaggtgtgcattccgaggtgcagctgktgsagtctgs

SEQ ID NO: 13 - DNA, 45 bp, synthetic construct
  misc_feature 1..45: note = SLIC-hu-VH6-for primer
  source 1..45: mol_type = other DNA
agcaacagctacaggtgtgcattcccaggtrcagctgcagsagtc

SEQ ID NO: 14 - DNA, 24 bp, synthetic construct
  misc_feature 1..24: note = hu-CH1gamma-rev primer
  source 1..24: mol_type = other DNA
gtccaccttggtgttgctgggctt

SEQ ID NO: 15 - DNA, 47 bp, synthetic construct
  misc_feature 1..47: note = SLIC-huVk2-for primer
  source 1..47: mol_type = other DNA
tagcaacagctacaggtgtgcattccgatgttgtgatgactcagtct

SEQ ID NO: 16 - DNA, 47 bp, synthetic construct
  misc_feature 1..47: note = SLIC-huVk3-for primer
  source 1..47: mol_type = other DNA
tagcaacagctacaggtgtgcattccgaaattgtgwtgacrcagtct

SEQ ID NO: 17 - DNA, 44 bp, synthetic construct
  misc_feature 1..44: note = SLIC-huVk5-for primer
  source 1..44: mol_type = other DNA
tagcaacagctacaggtgtgcattccgacatcgtgatgacccag

SEQ ID NO: 18 - DNA, 47 bp, synthetic construct
  misc_feature 1..47: note = SLIC-huVk7-for primer
  source 1..47: mol_type = other DNA
tagcaacagctacaggtgtgcattccgaaattgtgctgactcagtct

SEQ ID NO: 19 - DNA, 49 bp, synthetic construct
  misc_feature 1..49: note = SLIC-huVk8-for primer
  source 1..49: mol_type = other DNA
tagcaacagctacaggtgtgcattccgawrttgtgmtgackcagtctcc

SEQ ID NO: 20 - DNA, 47 bp, synthetic construct
  misc_feature 1..47: note = SLIC-huVk1long-for primer
  source 1..47: mol_type = other DNA
tagcaacagctacaggtgtgcattccgacatccrgwtgacccagtct

SEQ ID NO: 21 - DNA, 47 bp, synthetic construct
  misc_feature 1..47: note = SLIC-huVk2longw-for primer
  source 1..47: mol_type = other DNA
tagcaacagctacaggtgtgcattccgatrttgtgatgacycagwct

SEQ ID NO: 22 - DNA, 22 bp, synthetic construct
  misc_feature 1..22: note = huCk-rev primer
  source 1..22: mol_type = other DNA
acactctcccctgttgaagctc

SEQ ID NO: 23 - DNA, 44 bp, synthetic construct
  misc_feature 1..44: note = SLIC-huVl1-for primer
  source 1..44: mol_type = other DNA
tagcaacagctacaggtgtgcattcccagtctgtgytgackcag

SEQ ID NO: 24 - DNA, 44 bp, synthetic construct
  misc_feature 1..44: note = SLIC-huVl2-for primer
  source 1..44: mol_type = other DNA
tagcaacagctacaggtgtgcattcccagtctgccctgactcag

SEQ ID NO: 25 - DNA, 44 bp, synthetic construct
  misc_feature 1..44: note = SLIC-huVl3-for primer
  source 1..44: mol_type = other DNA
tagcaacagctacaggtgtgcattcctcctatgagctgaywcag

SEQ ID NO: 26 - DNA, 44 bp, synthetic construct
  misc_feature 1..44: note = SLIC-huVl4-for primer
  source 1..44: mol_type = other DNA
tagcaacagctacaggtgtgcattcccagcytgtgctgactcaa

SEQ ID NO: 27 - DNA, 44 bp, synthetic construct
  misc_feature 1..44: note = SLIC-huVl5-for primer
  source 1..44: mol_type = other DNA
tagcaacagctacaggtgtgcattcccagsctgtgctgactcag

SEQ ID NO: 28 - DNA, 44 bp, synthetic construct
  misc_feature 1..44: note = SLIC-huVl6-for primer
  source 1..44: mol_type = other DNA
tagcaacagctacaggtgtgcattccaattttatgctgactcag

SEQ ID NO: 29 - DNA, 44 bp, synthetic construct
  misc_feature 1..44: note = SLIC-huVl7-for primer
  source 1..44: mol_type = other DNA
tagcaacagctacaggtgtgcattcccagrctgtggtgactcag

SEQ ID NO: 30 - DNA, 44 bp, synthetic construct
  misc_feature 1..44: note = SLIC-huVl8-for primer
  source 1..44: mol_type = other DNA
tagcaacagctacaggtgtgcattcccagactgtggtgacccag

SEQ ID NO: 31 - DNA, 44 bp, synthetic construct
  misc_feature 1..44: note = SLIC-huVl9-for primer
  source 1..44: mol_type = other DNA
tagcaacagctacaggtgtgcattcccwgcctgtgctgactcag

SEQ ID NO: 32 - DNA, 44 bp, synthetic construct
  misc_feature 1..44: note = SLIC-huVlambda10-for primer
  source 1..44: mol_type = other DNA
tagcaacagctacaggtgtgcattcccaggcagggctgactcag

SEQ ID NO: 33 - DNA, 19 bp, synthetic construct
  misc_feature 1..19: note = huCl-1-rev primer
  source 1..19: mol_type = other DNA
tctccacggtgctcccttc

SEQ ID NO: 34 - DNA, 26 bp, synthetic construct
  misc_feature 1..26: note = huIg-PCR-vectorprimer-as
  source 1..26: mol_type = other DNA
ggaatgcacacctgtagctgttgcta

SEQ ID NO: 35 - DNA, 24 bp, synthetic construct
  misc_feature 1..24: note = huIg-PCR-vectorprimer-VH-s
  source 1..24: mol_type = other DNA
aagcccagcaacaccaaggtggac

SEQ ID NO: 36 - DNA, 26 bp, synthetic construct
  misc_feature 1..26: note = huIg-PCR-vectorprimer-as kappa
  source 1..26: mol_type = other DNA
ggaatgcacacctgtagctgttgcta

SEQ ID NO: 37 - DNA, 22 bp, synthetic construct
  misc_feature 1..22: note = huIg-PCR-vectorprimer-VK-s
  source 1..22: mol_type = other DNA
gagcttcaacaggggagagtgt

SEQ ID NO: 38 - DNA, 26 bp, synthetic construct
  misc_feature 1..26: note = huIg-PCR-vectorprimer-as lambda
  source 1..26: mol_type = other DNA
ggaatgcacacctgtagctgttgcta

SEQ ID NO: 39 - DNA, 19 bp, synthetic construct
  misc_feature 1..19: note = huIg-PCR-vectorprimer-VL-s
  source 1..19: mol_type = other DNA
gaagggagcaccgtggaga

SEQ ID NO: 40 - protein, 4 aa, Homo sapiens
EVQL

SEQ ID NO: 41 - protein, 4 aa, Homo sapiens
QVQL

SEQ ID NO: 42 - skipped

SEQ ID NO: 43 - protein, 4 aa, Homo sapiens
DIVM

SEQ ID NO: 44 - protein, 4 aa, Homo sapiens
DIQM

SEQ ID NO: 45 - protein, 5 aa, Homo sapiens
KLEIK